European Patent Specification EP 4 127 185 B1, published June 4, 2025. Title: HELPER FACTORS FOR EXPRESSING PROTEINS IN YEAST. Applicant: Lonza Ltd. The sequence listing filed with the application follows.

SEQUENCE LISTING (52 sequences)

SEQ ID NO: 1 - protein, 636 aa, Homo sapiens
EEEDKKEDVGTVVGIDLGTTYSCVGVFKNGRVEIIANDQGNRITPSYVAFTPEGERLIGDAAKNQLTSNPENTVFDAKRLIGRTWNDPSVQQDIKFLPFKVVEKKTKPYIQVDIGGGQTKTFAPEEISAMVLTKMKETAEAYLGKKVTHAVVTVPAYFNDAQRQATKDAGTIAGLNVMRIINEPTAAAIAYGLDKREGEKNILVFDLGGGTFDVSLLTIDNGVFEVVATNGDTHLGGEDFDQRVMEHFIKLYKKKTGKDVRKDNRAVQKLRREVEKAKRALSSQHQARIEIESFYEGEDFSETLTRAKFEELNMDLFRSTMKPVQKVLEDSDLKKSDIDEIVLVGGSTRIPKIQQLVKEFFNGKEPSRGINPDEAVAYGAAVQAGVLSGDQDTGDLVLLDVCPLTLGIETVGGVMTKLIPRNTVVPTKKSQIFSTASDNQPTVTIKVYEGERPLTKDNHLLGTFDLTGIPPAPRGVPQIEVTFEIDVNGILRVTAEDKGTGNKNKITITNDQNRLTPEEIERMVNDAEKFAEEDKKLKERIDTRNELESYAYSLKNQIGDKEKLGGKLSSEDKETMEKAVEEKIEWLESHQDADIEDFKAKKKELEEIVQPIISKLYGSAGPPPTGEEDTAEKDEL

SEQ ID NO: 2 - DNA, 1965 bp, Homo sapiens
atgaagctctccctggtggccgcgatgctgctgctgctcagcgcggcgcgggccgaggaggaggacaagaaggaggacgtgggcacggtggtcggcatcgacctggggaccacctactcctgcgtcggcgtgttcaagaacggccgcgtggagatcatcgccaacgatcagggcaaccgcatcacgccgtcctatgtcgccttcactcctgaaggggaacgtctgattggcgatgccgccaagaaccagctcacctccaaccccgagaacacggtctttgacgccaagcggctcatcggccgcacgtggaatgacccgtctgtgcagcaggacatcaagttcttgccgttcaaggtggttgaaaagaaaactaaaccatacattcaagttgatattggaggtgggcaaacaaagacatttgctcctgaagaaatttctgccatggttctcactaaaatgaaagaaaccgctgaggcttatttgggaaagaaggttacccatgcagttgttactgtaccagcctattttaatgatgcccaacgccaagcaaccaaagacgctggaactattgctggcctaaatgttatgaggatcatcaacgagcctacggcagctgctattgcttatggcctggataagagggagggggagaagaacatcctggtgtttgacctgggtggcggaaccttcgatgtgtctcttctcaccattgacaatggtgtcttcgaagttgtggccactaatggagatactcatctgggtggagaagactttgaccagcgtgtcatggaacacttcatcaaactgtacaaaaagaagacgggcaaagatgtcaggaaagacaatagagctgtgcagaaactccggcgcgaggtagaaaaggccaaacgggccctgtcttctcagcatcaagcaagaattgaaattgagtccttctatgaaggagaagacttttctgagaccctgactcgggccaaatttgaagagctcaacatggatctgttccggtctactatgaagcccgtccagaaagtgttggaagattctgatttgaagaagtctgatattgatgaaattgttcttgttggtggctcgactcgaattccaaagattcagcaactggttaaagagttcttcaatggcaaggaaccatcccgtggcataaacccagatgaagctgtagcgtatggtgctgctgtccaggctggtgtgctctctggtgatcaagatacaggtgacctggtactgcttgatgtatgtccccttacacttggtattgaaactgtgggaggtgtcatgaccaaactgattccaaggaacacagtggtgcctaccaagaagtctcagatcttttctacagcttctgataatcaaccaactgttacaatcaaggtctatgaaggtgaaagacccctgacaaaagacaatcatcttctgggtacatttgatctgactggaattcctcctgctcctcgtggggtcccacagattgaagtcacctttgagatagatgtgaatggtattcttcgagtgacagctgaagacaagggtacagggaacaaaaataagatcacaatcaccaatgaccagaatcgcctgacacctgaagaaatcgaaaggatggttaatgatgctgagaagtttgctgaggaagacaaaaagctcaaggagcgcattgatactagaaatgagttggaaagctatgcctattctctaaagaatcagattggagataaagaaaagctgggaggtaaactttcctctgaagataaggagaccatggaaaaagctgtagaagaaaagattgaatggctggaaagccaccaagatgctgacattgaagacttcaaagctaagaagaaggaactggaagaaattgttcaaccaattatcagcaaactctatggaagtgcaggccctcccccaactggtgaagaggatacagcagaaaaagatgagttgtag

SEQ ID NO: 3 - protein, 967 aa, Homo sapiens
LAVMSVDLGSESMKVAIVKPGVPMEIVLNKESRRKTPVIVTLKENERFFGDSAASMAIKNPKATLRYFQHLLGKQADNPHVALYQARFPEHELTFDPQRQTVHFQISSQLQFSPEEVLGMVLNYSRSLAEDFAEQPIKDAVITVPVFFNQAERRAVLQAARMAGLKVLQLINDNTATALSYGVFRRKDINTTAQNIMFYDMGSGSTVCTIVTYQMVKTKEAGMQPQLQIRGVGFDRTLGGLEMELRLRERLAGLFNEQRKGQRAKDVRENPRAMAKLLREANRLKTVLSANADHMAQIEGLMDDVDFKAKVTRVEFEELCADLFERVPGPVQQALQSAEMSLDEIEQVILVGGATRVPRVQEVLLKAVGKEELGKNINADEAAAMGAVYQAAALSKAFKVKPFVVRDAVVYPILVEFTREVEEEPGIHSLKHNKRVLFSRMGPYPQRKVITFNRYSHDFNFHINYGDLGFLGPEDLRVFGSQNLTTVKLKGVGDSFKKYPDYESKGIKAHFNLDESGVLSLDRVESVFETLVEDSAEEESTLTKLGNTISSLFGGGTTPDAKENGTDTVQEEEESPAEGSKDEPGEQVELKEEAEAPVEDGSQPPPPEPKGDATPEGEKATEKENGDKSEAQKPSEKAEAGPEGVAPAPEGEKKQKPARKRRMVEEIGVELVVLDLPDLPEDKLAQSVQKLQDLTLRDLEKQEREKAANSLEAFIFETQDKLYQPEYQEVSTEEQREEISGKLSAASTWLEDEGVGATTVMLKEKLAELRKLCQGLFFRVEERKKWPERLSALDNLLNHSSMFLKGARLIPEMDQIFTEVEMTTLEKVINETWAWKNATLAEQAKLPATEKPVLLSKDIEAKMMALDREVQYLLNKAKFTKPRPRPKDKNGTRAEPPLNASASDQGEKVIPPAGQTEDAEPISEPEKVETGSEPGDTEPLELGGPGAEPEQKEQSTGQKRPLKNDEL

SEQ ID NO: 4 - DNA, 3000 bp, Homo sapiens
atggcagacaaagttaggaggcagaggccgaggaggcgagtctgttgggccttggtggctgtgctcttggcagacctgttggcactgagtgatacactggcagtgatgtctgtggacctgggcagtgagtccatgaaggtggccattgtcaaacctggagtgcccatggaaattgtcttgaataaggaatctcggaggaaaacaccggtgatcgtgaccctgaaagaaaatgaaagattctttggagacagtgcagcaagcatggcgattaagaatccaaaggctacgctacgttacttccagcacctcctggggaagcaggcagataacccccatgtagctctttaccaggcccgcttcccggagcacgagctgactttcgacccacagaggcagactgtgcactttcagatcagctcgcagctgcagttctcacctgaggaagtgttgggcatggttctcaattattctcgttctctagctgaagattttgcagagcagcccatcaaggatgcagtgatcaccgtgccagtcttcttcaaccaggccgagcgccgagctgtgctgcaggctgctcgtatggctggcctcaaagtgctgcagctcatcaatgacaacaccgccactgccctcagctatggtgtcttccgccggaaagatattaacaccactgcccagaatatcatgttctatgacatgggctcaggcagcaccgtatgcaccattgtgacctaccagatggtgaagactaaggaagctgggatgcagccacagctgcagatccggggagtaggatttgaccgtaccctggggggcctggagatggagctccggcttcgagaacgcctggctgggcttttcaatgagcagcgcaagggtcagagagcaaaggatgtgcgggagaacccgcgtgccatggccaagctgctgcgtgaggctaatcggctcaaaaccgtcctcagtgccaacgctgaccacatggcacagattgaaggcctgatggatgatgtggacttcaaggcaaaagtgactcgtgtggaatttgaggagttgtgtgcagacttgtttgagcgggtgcctgggcctgtacagcaggccctccagagtgccgaaatgagtctggatgagattgagcaggtgatcctggtgggtggggccactcgggtccccagagttcaggaggtgctgctgaaggccgtgggcaaggaggagctggggaagaacatcaatgcagatgaagcagccgccatgggggcagtgtaccaggcagctgcgctcagcaaagcctttaaagtgaagccatttgtcgtccgagatgcagtggtctaccccatcctggtggagttcacgagggaggtggaggaggagcctgggattcacagcctgaagcacaataaacgggtactcttctctcggatggggccctaccctcaacgcaaagtcatcacctttaaccgctacagccatgatttcaacttccacatcaactacggcgacctgggcttcctggggcctgaagatcttcgggtatttggctcccagaatctgaccacagtgaagctaaaaggggtgggtgacagcttcaagaagtatcctgactacgagtccaagggcatcaaggctcacttcaacctggatgagagtggcgtgctcagtctagacagggtggagtctgtatttgagacactggtagaggacagcgcagaagaggaatctactctcaccaaacttggcaacaccatttccagcctgtttggaggcggtaccacaccagatgccaaggagaatggtactgatactgtccaggaggaagaggagagccctgcagaggggagcaaggacgagcctggggagcaggtggagctcaaggaggaagctgaggccccagtggaggatggctctcagcccccaccccctgaacctaagggagatgcaacccctgagggagaaaaggccacagaaaaagaaaatggggacaagtctgaggcccagaaaccaagtgagaaggcagaggcagggcctgagggcgtcgctccagccccagagggagagaagaagcagaagcccgccaggaagcggcgaatggtagaggagatcggggtggagctggttgttctggacctgcctgacttgccagaggataagctggctcagtcggtgcagaaacttcaggacttgacactccgagacctggagaagcaggaacgggaaaaagctgccaacagcttggaagcattcatatttgagacccaggacaagctgtaccagcccgagtaccaggaagtgtccacagaggagcagcgtgaggagatctctgggaagctcagcgccgcatccacctggctggaggatgagggtgttggagccaccacagtgatgttgaaggagaagctggctgagctgaggaagctgtgccaagggctgttttttcgggtagaggagcgcaagaagtggcccgaacggctgtctgccctcgataatctcctcaaccattccagcatgttcctcaagggggcccggctcatcccagagatggaccagatcttcactgaggtggagatgacaacgttagagaaagtcatcaatgagacctgggcctggaagaatgcaactctggccgagcaggctaagctgcccgccacagagaagcctgtgttgctctcaaaagacattgaagctaagatgatggccctggaccgagaggtgcagtatctgctcaataaggccaagtttaccaagccccggccccggcctaaggacaagaatgggacccgggcagagccacccctcaatgccagtgccagtgaccagggggagaaggtcatccctccagcaggccagactgaagatgcagagcccatttcagaacctgagaaagtagagactggatccgagccaggagacactgagcctttggagttaggaggtcctggagcagaacctgaacagaaagaacaatcgacaggacagaagcggcctttgaagaacgacgaactataa

SEQ ID NO: 5 - protein, 336 aa, Homo sapiens
GRDFYKILGVPRSASIKDIKKAYRKLALQLHPDRNPDDPQAQEKFQDLGAAYEVLSDSEKRKQYDTYGEEGLKDGHQSSHGDIFSHFFGDFGFMFGGTPRQQDRNIPRGSDIIVDLEVTLEEVYAGNFVEVVRNKPVARQAPGKRKCNCRQEMRTTQLGPGRFQMTQEVVCDECPNVKLVNEERTLEVEIEPGVRDGMEYPFIGEGEPHVDGEPGDLRFRIKVVKHPIFERRGDDLYTNVTISLVESLVGFEMDITHLDGHKVHISRDKITRPGAKLWKKGEGLPNFDNNNIKGSLIITFDVDFPKEQLTEEAREGIKQLLKQGSVQKVYNGLQGY

SEQ ID NO: 6 - DNA, 1077 bp, Homo sapiens
atggctccgcagaacctgagcaccttttgcctgttgctgctatacctcatcggggcggtgattgccggacgagatttctataagatcttgggggtgcctcgaagtgcctctataaaggatattaaaaaggcctataggaaactagccctgcagcttcatcccgaccggaaccctgatgatccacaagcccaggagaaattccaggatctgggtgctgcttatgaggttctgtcagatagtgagaaacggaaacagtacgatacttatggtgaagaaggattaaaagatggtcatcagagctcccatggagacattttttcacacttctttggggattttggtttcatgtttggaggaacccctcgtcagcaagacagaaatattccaagaggaagtgatattattgtagatctagaagtcactttggaagaagtatatgcaggaaattttgtggaagtagttagaaacaaacctgtggcaaggcaggctcctggcaaacggaagtgcaattgtcggcaagagatgcggaccacccagctgggccctgggcgcttccaaatgacccaggaggtggtctgcgacgaatgccctaatgtcaaactagtgaatgaagaacgaacgctggaagtagaaatagagcctggggtgagagacggcatggagtacccctttattggagaaggtgagcctcacgtggatggggagcctggagatttacggttccgaatcaaagttgtcaagcacccaatatttgaaaggagaggagatgatttgtacacaaatgtgacaatctcattagttgagtcactggttggctttgagatggatattactcacttggatggtcacaaggtacatatttcccgggataagatcaccaggccaggagcgaagctatggaagaaaggggaagggctccccaactttgacaacaacaatatcaagggctctttgataatcacttttgatgtggattttccaaaagaacagttaacagaggaagcgagagaaggtatcaaacagctactgaaacaagggtcagtgcagaaggtatacaatggactgcaaggatattga

SEQ ID NO: 7 - DNA, 1968 bp, Artificial Sequence
  codon-optimized nucleotide sequence
atgaagttgtccttggtcgctgctatgctgttgttgttgtctgctgctagagctgaggaagaggacaagaaagaggacgttggtactgttgttggtatcgacttgggtactacctactcctgtgtcggtgttttcaagaacggtagagtcgagattatcgctaacgaccaaggtaacagaatcaccccatcctacgttgctttcactccagagggtgagagattgattggtgacgctgctaagaaccaattgacctccaacccagagaacaccgttttcgacgctaagagattgatcggtagaacctggaacgacccatccgttcaacaagacatcaagttcttgccattcaaggtcgtcgagaagaagaccaagccttacatccaagttgacatcggtggtggtcaaactaagaccttcgctcctgaagagatctccgctatggttttgaccaagatgaaagaaaccgctgaggcttacttgggtaagaaggttactcacgctgttgttaccgtcccagcttacttcaacgacgctcaaagacaagctactaaggacgctggtactatcgctggtttgaacgtcatgagaatcatcaacgagccaaccgctgctgctattgcttacggtttggacaaaagagaaggagagaagaacatcttggttttcgacttgggtggtggtactttcgacgtttccttgttgactatcgacaacggtgttttcgaggtcgttgctaccaacggtgatactcacttgggtggtgaggacttcgaccaaagagttatggaacacttcatcaagttgtacaagaagaagactggtaaggacgtcagaaaggacaacagagctgtccaaaagttgagaagagaggtcgagaaggctaagagagctttgtcctctcaacaccaagctagaatcgagatcgagtccttctacgagggtgaggatttctctgagactttgaccagagctaagttcgaggaattgaacatggacttgttcagatccaccatgaagccagtccaaaaggttttggaggactccgacttgaagaagtctgacatcgacgagatcgttttggttggtggttctaccagaatcccaaagatccaacaattggtcaaagaattcttcaacggtaaagaaccatccagaggtatcaacccagacgaggctgttgcttacggtgctgctgttcaagctggtgttttgtctggtgaccaagacactggtgacttggttttgttggacgtctgtccattgaccttgggtatcgagactgttggtggtgtcatgaccaagttgatcccaagaaacaccgtcgtcccaactaagaagtcccaaatcttctctaccgcttccgacaaccaacctaccgttaccattaaggtttacgagggtgaaagaccattgactaaggacaaccacttgttgggtactttcgatttgactggtatcccaccagctccaagaggtgttccacaaatcgaggttactttcgagatcgacgtcaacggtatcttgagagttactgctgaggacaagggtactggtaacaagaacaagatcaccatcaccaacgaccaaaacagattgacccctgaagagattgagagaatggtcaacgacgctgagaagttcgctgaggaagataagaagttgaaagaaagaatcgacaccagaaacgagttggagtcctacgcttactccttgaagaaccaaatcggtgacaaagaaaagttgggaggtaagttgtcctccgaggataaagaaaccatggaaaaggctgtcgaagagaagatcgagtggttggagtctcaccaagacgctgacattgaggacttcaaggctaagaagaaagaattggaggaaatcgtccaacctatcatctccaagttgtacggttctgctggtccaccaccaactggtgaagaagatactgctgagaaggacgagttgtaatag

SEQ ID NO: 8 - DNA, 2907 bp, Artificial Sequence
  codon-optimized nucleotide sequence
ttggctgtcatgtctgttgacttgggttccgagtctatgaaggtcgctatcgttaagccaggtgtcccaatggaaatcgtcttgaacaaggaatccagaagaaagaccccagtcatcgtcaccttgaaggaaaacgagagattcttcggtgactccgctgcttctatggctatcaagaacccaaaggctaccttgagatacttccaacacttgttgggtaagcaagctgacaacccacacgtcgccttgtaccaagctagattcccagagcacgagttgactttcgacccacaaagacaaaccgtccacttccaaatctcttcccaattgcaattctccccagaggaagtcttgggtatggtcttgaactactccagatctttggctgaggacttcgctgagcaacctattaaggacgctgttatcaccgtcccagttttcttcaaccaggctgagagaagagctgtcttgcaagctgctagaatggctggtttgaaggtcttgcaattgatcaacgacaacaccgctaccgctttgtcctacggtgttttcagaagaaaggacatcaacaccaccgctcaaaacatcatgttctacgacatgggttctggttccaccgtctgtactatcgtcacctaccaaatggtcaagaccaaggaagctggtatgcaaccacaattgcaaatcagaggtgtcggtttcgacagaaccttgggtggtttggagatggaattgagattgagagagagattggctggtttgttcaacgagcaaagaaagggtcaaagagctaaggacgtcagagaaaacccaagagctatggctaagttgttgagagaggctaacagattgaagaccgtcttgtctgctaacgctgaccacatggctcaaatcgagggtttgatggacgacgttgacttcaaggctaaggttaccagagtcgagttcgaggaattgtgtgctgacttgttcgagagagttccaggtccagttcaacaagccttgcaatctgctgagatgtccttggacgagatcgagcaagttatcttggttggtggtgctaccagagtcccaagagttcaagaggttttgttgaaggctgtcggtaaggaagagttgggtaagaacattaacgctgacgaggctgctgctatgggtgctgtttaccaagctgctgctttgtccaaggctttcaaggttaagccattcgtcgtcagagatgctgtcgtctacccaatcttggttgagttcaccagagaggtcgaggaagaaccaggtatccactctttgaagcacaacaagagagtcttgttctccagaatgggtccatacccacaaagaaaggtcatcaccttcaacagatactcccacgacttcaacttccacatcaactacggtgacttgggtttcttgggtccagaggacttgagagttttcggttcccaaaacttgaccaccgtcaagttgaagggtgttggtgactccttcaagaagtacccagactacgagtccaagggtatcaaggctcacttcaacttggacgagtctggtgttttgtccttggacagagttgagtccgttttcgagactttggttgaggactctgctgaagaggaatccaccttgactaagttgggtaacaccatctcttccttgttcggtggtggtactactccagacgctaaggaaaacggtactgacaccgttcaagaggaagaggaatctccagctgagggttctaaggacgaaccaggtgagcaagttgagttgaaggaagaggctgaagctccagttgaggacggttctcaaccaccaccaccagaacctaagggtgatgctactccagaaggtgagaaggctactgagaaggaaaacggtgacaagtccgaggctcaaaagccatctgaaaaggctgaagctggtccagaaggtgttgctccagctcctgaaggtgaaaagaagcaaaagccagctagaaagagaagaatggtcgaagagatcggtgtcgagttggtcgttttggacttgccagatttgccagaggacaagttggctcaatccgtccaaaagttgcaagacttgaccttgagagacttggagaagcaagagagagagaaggctgctaactctttggaggctttcatcttcgagactcaagacaagttgtaccaacctgagtaccaagaggtttccaccgaggaacaaagagaggaaatctccggtaagttgtctgctgcttctacttggttggaggacgaaggtgttggtgctactaccgttatgttgaaggaaaagttggctgagttgagaaagttgtgtcaaggtttgttcttcagagtcgaagaaagaaagaagtggccagagagattgtccgctttggacaacttgttgaaccactcttccatgttcttgaagggtgctagattgatcccagagatggaccaaatcttcaccgaggttgagatgaccaccttggagaaggttatcaacgagacttgggcttggaagaacgctactttggctgagcaagctaagttgccagctaccgagaagccagttttgttgtctaaggacatcgaggctaagatgatggctttggacagagaggtccaatacttgttgaacaaggctaagttcaccaagccaagaccaagacctaaggacaagaacggtactagagctgagcctcctttgaacgcttctgcttctgaccaaggtgaaaaggttattccaccagctggtcaaactgaggacgctgagccaatttctgagccagagaaggttgagactggttctgaaccaggtgacactgagccattggaattgggtggtccaggtgctgaaccagagcaaaaggaacaatccactggtcaaaagagaccattgaagaacgacgagttgtaatag

SEQ ID NO: 9 - DNA, 1080 bp, Artificial Sequence
  codon-optimized nucleotide sequence
atggctccacaaaacttgtccactttctgtttgttgttgttgtacttgatcggtgctgttatcgctggtagagacttctacaagatcttgggtgttccaagatccgcttccatcaaggacatcaagaaggcttacagaaagttggctttgcaattgcacccagacagaaacccagacgacccacaagctcaagagaagttccaagatttgggtgctgcttacgaggttttgtctgactccgagaagagaaagcaatacgacacctacggtgaggaaggtttgaaggacggtcaccaatcttctcacggtgatatcttctcccacttcttcggtgacttcggtttcatgttcggtggtactccaagacaacaagacagaaacatcccaagaggttccgacatcatcgttgacttggaggttaccttggaggaagtctacgctggtaacttcgttgaggtcgtcagaaacaagccagtcgctagacaagctccaggtaagagaaagtgtaactgtagacaagagatgagaaccactcaattgggtccaggtagattccaaatgacccaagaggttgtctgtgacgagtgtccaaacgtcaagttggtcaacgaggaaagaaccttggaggttgagattgagccaggtgtcagagatggtatggaatacccattcattggtgagggtgagccacacgttgatggtgaaccaggtgacttgagattcagaatcaaggtcgtcaagcacccaatcttcgagagaagaggtgacgacttgtacaccaacgtcaccatttctttggtcgagtccttggtcggtttcgagatggacattactcacttggacggtcacaaggtccacatctctagagacaagattaccagaccaggtgctaagttgtggaagaagggtgagggtttgccaaacttcgataacaacaacatcaagggttccttgatcatcaccttcgacgtcgacttcccaaaggaacaattgaccgaggaagctagagagggtatcaagcaattgttgaagcaaggttccgtccaaaaggtctacaacggtttgcaaggttactaatag

SEQ ID NO: 10 - protein, 20 aa, Artificial Sequence
  Signal sequence
  MISC_FEATURE (3)..(3): X at position 3 is either F or L
  MISC_FEATURE (16)..(16): X at position 16 is either A or T
MKXSTNLILAIAAASXVVSA

SEQ ID NO: 11 - protein, 20 aa, Artificial Sequence
  Signal sequence
MKFSTNLILAIAAASAVVSA

SEQ ID NO: 12 - DNA, 60 bp, Artificial Sequence
  Signal sequence
atgaagttctccaccaatttgattctagctattgcagcagcttccgccgttgtctcagct

SEQ ID NO: 13 - protein, 36 aa, Artificial Sequence
  Leader sequence
  MISC_FEATURE (3)..(3): X at position 3 is either F or L
  MISC_FEATURE (16)..(16): X at position 16 is either A or T
MKXSTNLILAIAAASXVVSAAPVAPAEEAANHLHKR

SEQ ID NO: 14 - protein, 85 aa, Saccharomyces cerevisiae
MRFPSIFTAVLFAASSALAAPVNTTTEDETAQIPAEAVIGYSDLEGDFDVAVLPFSNSTNNGLLFINTTIASIAAKEEGVSLEKR

SEQ ID NO: 15 - protein, 18 aa, Homo sapiens
MKLSLVAAMLLLLSAARA

SEQ ID NO: 16 - protein, 32 aa, Homo sapiens
MADKVRRQRPRRRVCWALVAVLLADLLALSDT

SEQ ID NO: 17 - protein, 45 aa, Saccharomyces cerevisiae
MFFNRLSAGKLLVPLSVVLYALFVVILPLQNSFHSSNVLVRGADD

SEQ ID NO: 18 - DNA, 135 bp, Saccharomyces cerevisiae
atgtttttcaacagactaagcgctggcaagctgctggtaccactctccgtggtcctgtacgcccttttcgtggtaatattacctttacagaattctttccactcctccaatgttttagttagaggtgccgatgat

SEQ ID NO: 19 - protein, 22 aa, Homo sapiens
MAPQNLSTFCLLLLYLIGAVIA

SEQ ID NO: 20 - protein, 4 aa, Homo sapiens
KDEL

SEQ ID NO: 21 - protein, 4 aa, Homo sapiens
NDEL

SEQ ID NO: 22 - protein, 4 aa, Homo sapiens
RDEL

SEQ ID NO: 23 - protein, 4 aa, Homo sapiens
DDEL

SEQ ID NO: 24 - DNA, 491 bp, Pichia pastoris
cttttttgtagaaatgtcttggtgtcctcgtccaatcaggtagccatctctgaaatatctggctccgttgcaactccgaacgacctgctggcaacgtaaaattctccggggtaaaacttaaatgtggagtaatggaaccagaaacgtctcttcccttctctctccttccaccgcccgttaccgtccctaggaaattttactctgctggagagcttcttctacggcccccttgcagcaatgctcttcccagcattacgttgcgggtaaaacggaggtcgtgtacccgacctagcagcccagggatggaaaagtcccggccgtcgctggcaataatagcgggcggacgcatgtcatgagattattggaaaccaccagaatcgaatataaaaggcgaacacctttcccaattttggtttctcctgacccaaagactttaaatttaatttatttgtccctatttcaatcaattgaacaactatcacctgcaggcc

SEQ ID NO: 25 - DNA, 488 bp, Pichia pastoris
cttttttgtagaaatgtcttggtgtcctcgtccaatcaggtagccatctctgaaatatctggctccgttgcaactccgaacgacctgctggcaacgtaaaattctccggggtaaaacttaaatgtggagtaatggaaccagaaacgtctcttcccttctctctccttccaccgcccgttaccgtccctaggaaattttactctgctggagagcttcttctacggcccccttgcagcaatgctcttcccagcattacgttgcgggtaaaacggaggtcgtgtacccgacctagcagcccagggatggaaaagtcccggccgtcgctggcaataatagcgggcggacgcatgtcatgagattattggaaaccaccagaatcgaatataaaaggcgaacacctttcccaattttggtttctcctgacccaaagactttaaatttaatttatttgtccctatttcaatcaattgaacaactatcaaaacaca

SEQ ID NO: 26 - DNA, 985 bp, Pichia pastoris
agggcatcattgaggtttccacaaaaggaagaaacatggatccagagacatcaacagagaggaaagcgggtagtgaagccgaagccacaacacagcccgatttggaagggagttcacaatcaaggtgagtccagccattttttttcttttttttttttttattcaggtgaacccacctaactatttttaactgggatccagtgagctcgctgggtgaaagccaaccatcttttgtttcggggaaccgtgctcgccccgtaaagttaatttttttttcccgcgcagctttaatctttcggcagagaaggcgttttcatcgtagcgtgggaacagaataatcagttcatgtgctatacaggcacatggcagcagtcactattttgctttttaaccttaaagtcgttcatcaatcattaactgaccaatcagattttttgcatttgccacttatctaaaaatacttttgtatctcgcagatacgttcagtggtttccaggacaacacccaaaaaaaggtatcaatgccactaggcagtcggttttatttttggtcacccacgcaaagaagcacccacctcttttaggttttaagttgtgggaacagtaacaccgcctagagcttcaggaaaaaccagtacctgtgaccgcaattcaccatgatgcagaatgttaatttaaacgagtgccaaatcaagatttcaacagacaaatcaatcgatccatagttacccattccagccttttcgtcgtcgagcctgcttcattcctgcctcaggtgcataactttgcatgaaaagtccagattagggcagattttgagtttaaaataggaaatataaacaaatataccgcgaaaaaggtttgtttatagcttttcgcctggtgccgtacggtataaatacatactctcctcccccccctggttctctttttcttttgttacttacattttaccgttccgtcactcgcttcactcaacaacaaaa

SEQ ID NO: 27 - DNA, 1001 bp, Pichia pastoris
catgttggtattgtgaaatagacgcagatcgggaacactgaaaaataacagttattattcgagatctaacatccaaagacgaaaggttgaatgaaacctttttgccatccgacatccacaggtccattctcacacataagtgccaaacgcaacaggaggggatacactagcagcagaccgttgcaaacgcaggacctccactcctcttctcctcaacacccacttttgccatcgaaaaaccagcccagttattgggcttgattggagctcgctcattccaattccttctattaggctactaacaccatgactttattagcctgtctatcctggcccccctggcgaggttcatgtttgtttatttccgaatgcaacaagctccgcattacacccgaacatcactccagatgagggctttctgagtgtggggtcaaatagtttcatgttccccaaatggcccaaaactgacagtttaaacgctgtcttggaacctaatatgacaaaagcgtgatctcatccaagatgaactaagtttggttcgttgaaatgctaacggccagttggtcaaaaagaaacttccaaaagtcggcataccgtttgtcttgtttggtattgattgacgaatgctcaaaaataatctcattaatgcttagcgcagtctctctatcgcttctgaaccccggtgcacctgtgccgaaacgcaaatggggaaacacccgctttttggatgattatgcattgtctccacattgtatgcttccaagattctggtgggaatactgctgatagcctaacgttcatgatcaaaatttaactgttctaacccctacttgacagcaatatataaacagaaggaagctgccctgtcttaaacctttttttttatcatcattattagcttactttcataattgcgactggttccaattgacaagcttttgattttaacgacttttaacgacaacttgagaagatcaaaaaacaactaattattcgaaacg

SEQ ID NO: 28 - DNA, 1000 bp, Pichia pastoris
gcttaaaggactccatttcctaaaatttcaagcagtcctctcaactaaatttttttccattcctctgcacccagccctcttcatcaaccgtccagccttctcaaaagtccaatgtaagtagcctgcaaattcaggttacaacccctcaattttccatccaagggcgatccttacaaagttaatatcgaacagcagagactaagcgagtcatcatcaccacccaacgatggtgaaaaactttaagcatagattgatggagggtgtatggcacttggcggctgcattagagtttgaaactatggggtaatacatcacatccggaactgatccgactccgagatcatatgcaaagcacgtgatgtaccccgtaaactgctcggattatcgttgcaattcatcgtcttaaacagtacaagaaactttattcatgggtcattggactctgatgaggggcacatttccccaatgattttttgggaaagaaagccgtaagaggacagttaagcgaaagagacaagacaacgaacagcaaaagtgacagctgtcagctacctagtggacagttgggagtttccaattggttggttttgaatttttacccatgttgagttgtccttgcttctccttgcaaacaatgcaagttgataagacatcaccttccaagataggctatttttgtcgcataaatttttgtctcggagtgaaaaccccttttatgtgaacagattacagaagcgtcctacccttcaccggttgagatggggagaaaattaagcgatgaggagacgattattggtataaaagaagcaaccaaaatcccttattgtccttttctgatcagcatcaaagaatattgtcttaaaacgggcttttaactacattgttcttacacattgcaaacctcttccttctatttcggatcaactgtattgactacattgatcttttttaacgaagtttacgacttactaaatccccacaaacaaatcaactgagaaaa

SEQ ID NO: 29 - DNA, 975 bp, Pichia pastoris
gtagcttgggtaggacttgacaagtacggcttccgtggtcataccaaacgcctttgttaccgttggctatacctaatgaccaaggcatttgtggattataacggtatcgtagttgaaaaatatgacgtaaccactggtactagcccccacaaggttgatgctgaatacgggaatcaaggtgccgattttaaaggagtagccactgaagggtttggctgggtcaatgcctcttttattttgggattaacctacttagatgtccaaggcatccgtgcgataggcgccgttacgtcccctgatgtatttttcaggaagctcaaaccttgggaacgcgcaagttatggcctaaggccatgtaacgagatagtcaagtcaaactagaagtatacggtttccccgcagaaatagcagaaataggcgacaaatacatacaacattttcattgtgatagggggcggcggttcctaggagggacaacccccagaaaccttgtagactacgttttcacgacgatgggttattactgtaaaggaagaatatactacccaccagttgaatgtttgaacggatcaaaggtcgaagggagtacacggcccaaccaacgtagctaccggagaaagcaagactttcccaaaccaaatagctccgggtttcttctccggcaacccgtcagtttttgtgtggccggacaaaaattcgcaccctcagtctaattgaaaggtcgggctccgagctctaggcgtttgcgcatgtaatattgcatcccctcccatagataatactgcgcgaacacagggtgcaaattatgatgaccacacatgccagtgaccaaaacagttttttagtctttaaaaaccctcggaacttctgagtatataaaggcttctcatttcctacaagcaaacaaagaagaaacttccactttctaactttttatctatagactttagagttacaaccaacgaacaataacaa

SEQ ID NO: 30 - DNA, 699 bp, Pichia pastoris
cgcattatttgggtcggctactgtcattggttatgatggccttaccgagcacgaaggtggttggatagaccacaactggaaacagttgtacaaacagattgcattcatttttgcttgtattggatactcgatggccatcaccgctcttatctgtttcatcctcaaccgtattccatttttgcaactgcgagcttcagaagaggctgaggagaaaggtatggatgaggatcagattggagagttcgcttatgactacgtggaagtacgtcgtgattttttggcttggggatcaggcccaaacaatggcttcaaggagccggaagttctggatcaggtagttccggttaatgatttcagcagtgaccagaatgtgactaatcagaccaacgaatctgagaagcagtagagtaaatatagagatgatatttagtgtattctaatgcttatgtaatgtattaagcaaaaagttgtgtttatgagttagcatttgtcttagcaaacataaaattatgtcgacatttgcaacccgcatgtctagtgtttttagatcgatcttcgatgtgtagaataatgcctccacgtgatgccccgcgattttgttgggtcgcaatgcctccaacataaacccatcacgtataaaaagccctcttaaccctcccccctgtttcgtttgcttcatcacttaacctgaactatcaa

SEQ ID NO: 31 - DNA, 991 bp, Pichia pastoris
gcaaggcaactgagaaattgaatagtggtttcaagcccgctgactttttgtattatctcaatgtcggtgtttcacagtccccagaagggggctttgccttcaagggagacggaagagacatcgtcaaccctggggagaagtatttcaaatggcgcaagttcgctaatttttacgattaagcagtgctgtatggggtagttaataaatcgggaatatccttctgacgtgactgtaacaaatctctttttacgtggtgcgcatactggacagaggcagagtctcaatttcttcttttgagacaggctactacagcctgtgattcctcttggtacttggatttgcttttatctggctccgttgggaactgtgcctgggttttgaagtatcttgtggatgtgtttctaacactttttcaatcttcttggagtgagaatgcaggactttgaacatcgtctagctcgttggtaggtgaaccgttttaccttgcatgtggttaggagttttctggagtaaccaagaccgtcttatcatcgccgtaaaatcgctcttactgtcgctaataatcccgctggaagagaagttcgaacagaagtagcacgcaaagctcttgtcaaatgagaattgttaatcgtttgacaggtcacactcgtgggctatgtacgatcaacttgccggctgttgctggagagatgacaccagttgtggcatggccaattggtattcagccgtaccactgtatggaaaatgagattatcttgttcttgatctagtttcttgccattttagagttgccacattcgtaggtttcagtaccaataatggtaacttccaaacttccaacgcagataccagagatctgccgatccttccccaacaataggagcttactacgccatacatatagcctatctattttcactttcgcgtgggtgcttctatataaacggttccccatcttccgtttcatactacttgaattttaagcactaaa

SEQ ID NO: 32 - DNA, 864 bp, Pichia pastoris
cttttctttgggcaaggaaaaatcaagaaaaagcagaggttaaagttttcaggggaatggcaattgctttatatatgggagaaagttaactacgtcggtgctgtaggcgtagagagcgactggagaatgcgtgatgaggtcgtctcttttcgcccccccttggcggggtaaaaattgcactactgcagaattactacacccctattccgaggagacggagtgcgacaaaaatggtaaagttcaccctagtctgcgacttttaattgacggacaccggcgtttacatgcgaaaaaaactaaagtgcgcgcatttcacggccgaggggggtcccacttgggactgagagggggtgggatctgaaatcgaggaggtatcaagaccccccgtttctcaactccctaatcaaaaattacgaagtcctcgttggaaaggagttaaaataattaagcggggtcggacgccataccgaggttatcttgcaggcattttactaatattggaattcggagctcaacttgcaaccaggcagggtttagctatgtaatcaatgtaatcaatataataaagcactaccacatcgaaggtttgggagggaggccaatagtgtcccccacagggtgctgatatcgcgattcttgggtgaggagacacatatttcactcctctcaccaaccaaccaagcggctcctcgcaagatgatttatccgattatccggacactatactcccatccagtttgatgccgatttcatcgattgtcctaaataatccttaaatatgtatagaacggtaccctggggttacataatccttatttaataatccctcccccaccgcttttctttttttttcttcttattgtc

SEQ ID NO: 33 - DNA, 1000 bp, Pichia pastoris
aaatggcagaaggatcagcctggacgaagcaaccagttccaactgctaagtaaagaagatgctagacgaaggagacttcagaggtgaaaagtttgcaagaagagagctgcgggaaataaattttcaatttaaggacttgagtgcgtccatattcgtgtacgtgtccaactgttttccattacctaagaaaaacataaagattaaaaagataaacccaatcgggaaactttagcgtgccgtttcggattccgaaaaacttttggagcgccagatgactatggaaagaggagtgtaccaaaatggcaagtcgggggctactcaccggatagccaatacattctctaggaaccagggatgaatccaggtttttgttgtcacggtaggtcaagcattcacttcttaggaatatctcgttgaaagctacttgaaatcccattgggtgcggaaccagcttctaattaaatagttcgatgatgttctctaagtgggactctacggctcaaacttctacacagcatcatcttagtagtcccttcccaaaacaccattctaggtttcggaacgtaacgaaacaatgttcctctcttcacattgggccgttactctagccttccgaagaaccaataaaagggaccggctgaaacgggtgtggaaactcctgtccagtttatggcaaaggctacagaaatcccaatcttgtcgggatgttgctcctcccaaacgccatattgtactgcagttggtgcgcattttagggaaaatttaccccagatgtcctgattttcgagggctacccccaactccctgtgcttatacttagtctaattctattcagtgtgctgacctacacgtaatgatgtcgtaacccagttaaatggccgaaaaactatttaagtaagtttatttctcctccagatgagactctccttcttttctccgctagttatcaaactataaacctattttacctcaaatacctccaacatcacccacttaaaca

SEQ ID NO: 34 - DNA, 549 bp, Pichia pastoris
aatgatataaacaacaattgagtgacaggtctactttgttctcaaaaggccataaccatctgtttgcatctcttatcaccacaccatcctcctcatctggccttcaattgtggggaacaactagcatcccaacaccagactaactccacccagatgaaaccagttgtcgcttaccagtcaatgaatgttgagctaacgttccttgaaactcgaatgatcccagccttgctgcgtatcatccctccgctattccgccgcttgctccaaccatgtttccgcctttttcgaacaagttcaaatacctatctttggcaggacttttcctcctgccttttttagcctcaggtctcggttagcctctaggcaaattctggtcttcatacctatatcaacttttcatcagatagcctttgggttcaaaaaagaactaaagcaggatgcctgatatataaatcccagatgatctgcttttgaaactattttcagtatcttgattcgtttacttacaaacaactattgttgattttatctggagaataatcgaacaaa

SEQ ID NO: 35 - DNA, 1000 bp, Pichia pastoris
attactgttttgggcaatcctgttgataagacgcattctagagttgtttcatgaaagggttacgggtgttgattggtttgagatatgccagaggacagatcaatctgtggtttgctaaactggaagtctggtaaggactctagcaagtccgttactcaaaaagtcataccaagtaagattacgtaacacctgggcatgactttctaagttagcaagtcaccaagagggtcctatttaacgtttggcggtatctgaaacacaagacttgcctatcccatagtacatcatattacctgtcaagctatgctaccccacagaaataccccaaaagttgaagtgaaaaaatgaaaattactggtaacttcaccccataacaaacttaataatttctgtagccaatgaaagtaaaccccattcaatgttccgagatttagtatacttgcccctataagaaacgaaggatttcagcttccttaccccatgaacagaaatcttccatttaccccccactggagagatccgcccaaacgaacagataatagaaaaaagaaattcggacaaatagaacactttctcagccaattaaagtcattccatgcactccctttagctgccgttccatccctttgttgagcaacaccatcgttagccagtacgaaagaggaaacttaaccgataccttggagaaatctaaggcgcgaatgagtttagcctagatatccttagtgaagggttgttccgatacttctccacattcagtcatagatgggcagctttgttatcatgaagagacggaaacgggcattaagggttaaccgccaaattatataaagacaacatgtccccagtttaaagtttttctttcctattcttgtatcctgagtgaccgttgtgtttaatataacaagttcgttttaacttaagaccaaaaccagttacaacaaattataacccctctaaacactaaagttcactcttatcaaactatcaaacatcaaaa

SEQ ID NO: 36 - DNA, 1000 bp, Pichia pastoris
gtcaactgcgtactcttttgtcgaatggactactgaatctgcctcgatagccactataggaaggtccatagaggccagtttttcaactagtcttggtggaaagaaaccgacaaagcctttcatggagtcaccgatactgaaaggttcaaacaaagaatgcttgggtagtctcttaatacccatggcaacgaaaaaggggtcttcattgttcaacatgaattcgtatccacctttaatgtagtcataaagctgctgaagttccgaatcagtgatggaactgtctacagtgacaatataggagttctcaatcaccttatatccagtcgaatatatctggatagggtcgggtctcactgtggaagattcaaatgggttagatccctgtaatttcagcgatggagactcagtatgatggggcaaggaaaacggcaattggatattcaattggtcaagagatggtatcaaaagcgagtgtgccagggtagccacggtagccactgatgctaatctgataattttcatttctggagtgtcaaaacagtagtgataaaaggctatgaaggaggttgtctaggggctcgcggaggaaagtgattcaaacagacctgccaaaaagagaaaaaagagggaatccctgttctttccaatggaaatgacgtaactttaacttgaaaaataccccaaccagaagggttcaaactcaacaaggattgcgtaattcctacaagtagcttagagctgggggagagacaactgaaggcagcttaacgataacgcggggggattggtgcacgactcgaaaggaggtatcttagtcttgtaacctcttttttccagaggctattcaagattcataggcgatatcgatgtggagaagggtgaacaatataaaaggctggagagatgtcaatgaagcagctggatagatttcaaattttctagatttcagagtaatcgcacaaaacgaaggaatcccaccaagcaaaaaaaaaaatctaag

SEQ ID NO: 37 - DNA, 704 bp, Pichia pastoris
aaattaatccataagataaggcaaatgtgcttaagtaattgaaaacagtgttgtgattatataagcatggtatttgaatagaactactggggttaacttatctagtaggatggaagttgagggagatcaagatgcttaaagaaaaggattggccaatatgaaagccataattagcaatacttatttaatcagataattgtggggcattgtgacttgacttttaccaggacttcaaacctcaaccatttaaacagttatagaagacgtaccgtcacttttgcttttaatgtgatctaaatgtgatcacatgaactcaaactaaaatgatatcttttactggacaaaaatgttatcctgcaaacagaaagctttcttctattctaagaagaacatttacattggtgggaaacctgaaaacagaaaataaatactccccagtgaccctatgagcaggatttttgcatccctattgtaggcctttcaaactcacacctaatatttcccgccactcacactatcaatgatcacttcccagttctcttcttcccctattcgtaccatgcaacccttacacgccttttccatttcggttcggatgcgacttccagtctgtggggtacgtagcctattctcttagccggtatttaaacatacaaattcacccaaattctaccttgataaggtaattgattaatttcataaat

SEQ ID NO: 38 - DNA, 1000 bp, Pichia pastoris
agctcagattggaaatgatttttgatcctaccaagaagcctttgatttccagaatctccgctaagtaagtaacccccgcaaacgcatgcatccatgcaaacaaaatactaacaattttagccccgttgttgagaaacccagaaaattgaatgttcaaccaatccagacgatcaataagaaaaaaggcccaaaggctacttccaaacctgctgccgccaaacctgctccttcaaaagccggtcccaagggaggtaagaaggtgagaaagccaaagaagacagttgaagaattggatcaggaaatggctgactactttgaaaataagaattagcccaacaaaatatgtacaagtattatataaatgaatctacatggtgtgttttatttagatcctccaaaccaaggaaagaaactaaacttatctccggacttacgagtcaaataactatccgcagttccttggaactcagactttcttccataagcggtcatatcatctttggactgtgggaatcctggacgaatctttgaaatgtcataatcttgctctctatctccaagcacagcgtccggtaaatgctggttcttctttctcagatgaatcttggatttaacaaataaagccgtgcctatggctaatgtactcaaaaacaaagtctgcttccagaatttcgcaaacgatggaatgccatttcctgtaaatgtactcattgaacctatgtttgattaaagttggtgtgaagtcatcaaacgagagtaaaatcagatactcgtgcaccggccaaaattgactgagctaatctctgcaggcttgacatccgaacacaacaaataggcgacaaatcttaactatctaatcgtaggctatggtagaactttgtgggggtagaggaagactacaacagcaagacaaaacaaaagagtcatagtttgactctctgcttttttcttctttctcttctttttcttcctccatattcgttatttatttcgaactgga

SEQ ID NO: 39 - DNA, 1000 bp, Pichia pastoris
cagccattaatctcacctcagtttttgaatcagtagaatttttaatgaaacaaacggttggtatattatttgatagagttgccaaatttccaaagataaatttttcatcaggtaatatcctgaataccgtaacatagtgactattggaagacactgctatcatattatatttcggataaaaatccaaaccccagaccgacctcttgagtctcaactccaagtcagccgcaactttaattatccgtggattgggagctagtttggacaacgcatcagtataatataactttacggttccattatcagacgctattgcaagaacttcctttccattgatctcgccaatgcggcagtaattgatatcgtagggtaggtctggaaagacgctggcgcttgtgtcccattctgcaggaatctctggcacggtgctaatggtagttatccaacggagctgaggtagtcgatatatctggatatgccgcctataggataaaaacaggagagggtgaaccttgcttatggctactagattgttcttgtactctgaattctcattatgggaaactaaactaatctcatctgtgtgttgcagtactattgaatcgttgtagtatctacctggagggcattccatgaattagtgagataacagagttgggtaactagagagaataatagacgtatgcatgattactacacaacggatgtcgcactctttccttagttaaaactatcatccaatcacaagatgcgggctggaaagacttgctcccgaaggataatcttctgcttctatctcccttcctcatatggtttcgcagggctcatgccccttcttccttcgaactgcccgatgaggaagtccttagcctatcaaagaattcgggaccatcatcgatttttagagccttacctgatcgcaatcaggatttcactactcatataaatacatcgctcaaagctccaactttgcttgttcatacaattcttgatattcaca

SEQ ID NO: 40 - DNA, 1000 bp, Pichia pastoris
tggttccctctcggtccaataccaaaaatattatcaccatacaggtctcccttcgataccagtgcaaagttgaaccgtgggattaccttggaatctacaaaaatagtgtcactcacaagtttgtcatcaaccacgctgccgcttgcaaaggagaactgaacatgaaggttgttagggtttgttatattggaataagtggtggatttgttgaaggcgaacgcaccaaagctacatccgtcctgagcacactgtgaatttgtcacggaattgaccaagaggtcagacgatcctgtatcccattgagccgttatgctttgtgggggaaaccctatttctatcgtactaagaaaaccaatggtgaactcatattcggtatcaatggcgacgattccagcatagcctgtagacagtaacaacactagggcaacagcaactaacatatcttcattgatgaaacgttgtgatcggtgtgacttttatagtaaaagctacaactgtttgaaataccaagatatcattgtgaatggctcaaaagggtaatacatctgaaaaacctgaagtgtggaaaattccgatggagccaactcatgataacgcagaagtcccattttgccatcttctcttggtatgaaacggtagaaaatgatccgagtatgccaattgatactcttgattcatgccctatagtttgcgtagggtttaattgatctcctggtctatcgatctgggacgcaatgtagaccccattagtggaaacactgaaagggatccaacactctaggcggacccgctcacagtcatttcaggacaatcaccacaggaatcaactacttctcccagtcttccttgcgtgaagcttcaagcctacaacataacacttcttacttaatctttgattctcgaattgtttacccaatcttgacaacttagcctaagcaatactctggggttatatatagcaattgctcttcctcgctgtagcgttcattccatctttcta

SEQ ID NO: 41 - DNA, 1001 bp, Pichia pastoris
gatatcgatctacacttaatagtagatgacgaggcatctctccaataggtaccatatctggtgtttcttgtaatttaagaatctgttggtctatgaatgtagatttgtcatgaacaatgatatatgggtcaggaggacaagatggtttctctgagttgggttgttgaggtgcctggcaagacttcggagcgttgatatccccaagacttgtagtgaccgatagttgaagcgtgtgtttgcaggaacggcacatcaatgcaactttcgtaactttggaattgagagttgatgcactgatgacgatacccgaaattttgacgattttaccaatatgacttgaagacaagtctctcattgaaaccttattatcgttactaagcaaaacgagctgacaagaagggaaggtggtcggtatttcctcgttgttcaaatatatgattctcctggcaatatctgtgatggcctgttcaaaaagtggaatcatttctgcaggatcatctaccaactttttattgagctcctcattgaatacgattaagtggtcattttgaatcgtcagtaagtacttgtttacaagtaaattctgtctgagttgttctctgtagatgtactgattttccatacgaaactccaaaatgaacgaacggaatgccttaatgacctcactgaactggtcatcgttctgttctccgggaaggacacttgtgttaaagactgatgctctatcaaaggacattgcaacaaagtataaacggttgtgagcgggaaaaagatgtgtaggtaattgtcgtagatgagactgattcagtagaaaacgcgtcctgcactatttttttctttcttcattacatttcctaatcgggacaaaatgaatctaaagacgtggttatgtagtacacgcatcgataggctatccccataccaaaacactattttaccccatccttgacaggttataaatatgcgatagtatgagtatcttcaaattcagctgaaatatc

SEQ ID NO: 42 - DNA, 1000 bp, Pichia pastoris
aataaaaaaacgttatagaaagaaattggactacgatatgctccaatccaaattgtcaaaattgaccaccgaaaaagaacaattggaatttgacaagaggaacaactcactagattctcaaacggagcgtcacctagagtcagtttccaagtcaattacagaaagtttggaaacagaagaggagtatctacaattgaattccaaacttaaagtcgagctgtccgaattcatgtcgctaaggctttcttacttggaccccatttttgaaagtttcattaaagttcagtcaaaaattttcatggacatttatgacacattaaagagcggactaccttatgttgattctctatccaaagaggattatcagtccaagatcttggactctagaatagataacattctgtcgaaaatggaagcgctgaaccttcaagcttacattgatgattagagcaatgatataaacaacaattgagtgacaggtctactttgttctcaaaaggccataaccatctgtttgcatctcttatcaccacaccatcctcctcatctggccttcaattgtggggaacaactagcatcccaacaccagactaactccacccagatgaaaccagttgtcgcttaccagtcaatgaatgttgagctaacgttccttgaaactcgaatgatcccagccttgctgcgtatcatccctccgctattccgccgcttgctccaaccatgtttccgcctttttcgaacaagttcaaatacctatctttggcaggacttttcctcctgccttttttagcctcaggtctcggttagcctctaggcaaattctggtcttcatacctatatcaacttttcatcagatagcctttgggttcaaaaaagaactaaagcaggatgcctgatatataaatcccagatgatctgcttttgaaactattttcagtatcttgattcgtttacttacaaacaactattgttgattttatctggagaataatcgaacaaa

SEQ ID NO: 43 - DNA, 1000 bp, Pichia pastoris
attgttgtgaatactctccttcatttggatttcttggacttcggactctcttgatctctcttcgaaagttttaactctgttcatgtataattttacccgctgtaggtcgctcataataccatgagtatgcacatcttttactccattaactttcaggtatgcaaaatacaatgaagatagtatatagctcaaagaatttagcattttgcattgatctaattgtgacattttctctatgatatcatctagcttcttaaactcgagaatctcgtccaacgaggcagaaacattgtccagtcttacgtcaagattattcacgagtttctggaccgtatcaacgttttccatcttaagattacagtaagtatcgtccttttgaactgcaaaggtagaaaagttaatttttgatttggtagtacactatgaaacttgctcaccccaatctttcctcctgacaggttgatctttatccctctactaaattgccccaagtgtatcaagtagactagatctcgcgaaagaacagcctaataaactccgaagcatgatggcctctatccggaaaacgttaagagatgtggcaacaggagggcacatagaatttttaaagacgctgaagaatgctatcatagtccgtaaaaatgtgatagtactttgtttagtgcgtacgccacttattcggggccaatagctaaacccaggtttgctggcagcaaattcaactgtagattgaatctctctaacaataatggtgttcaatcccctggctggtcacggggaggactatcttgcgtgatccgcttggaaaatgttgtgtatccctttctcaattgcggaaagcatctgctacttcccataggcaccagttacccaattgatatttccaaaaaagattaccatatgttcatctagaagtataaatacaagtggacattcaatgaatatttcattcaattagtcattgacactttcatcaacttactacgtcttattcaacaat

SEQ ID NO: 44 - DNA, 1000 bp, Pichia pastoris
tatacggtctatccactttggaaacgatgtagttgaaacggggaagtaatagtggttcccaaacgacatgaagaggttatataagtttgcaagagggtgacaccattttagttgtggttcccgggtatttttttaatctttttagtctaagatagcctccccagatattaccgagttgggccatttggggcggtatcggtggtatctgatggtagcgcgtttttacatgcctgtgcattgaactggcaaagagtatactatcgtggggccctgaaggaggcagcaaatggaccgtcaattggttgatcagggactcaagacaggtattgagcttttcaaacaaaaagagtataggcgctgctacaaggcatttacttctactatcaatttcattgagaatgatcccgagttggccgccagctgtgtatctcaactgatatctctgttagattgtagggcagcctgtttggaaaagctagatcaattgaatatggccttgaaagatggtcttaaaatgatcaagagagagtgccacaactgcaagggttatttgagaacttgcaaaattttagacctacaagggaagatcagtgaggctttgtctacagcaagagaagggatctccataatagaaactagaagagatcaggataatcaatttagatattccaaggttcttttggaacaattaaaggaactgaaaaatgcactgaaaatcaaattggacaagaaaaatcagctacacttcaaagttttaaagtttgacgcaccagtgccttgtacaaagaaactaagattagtcactccaagaacaatagatccttccatttttttgccgatagagctagtgaagctgatctttcgcctgttgaatttctcagacatgtatgcctgtttattggtctcaacaaaatggaactcaattatatcctcatcaccggaactgtttcgaaaacttcagttgaaatcccaactgtccaacaaggcgttaaacaattgt

SEQ ID NO: 45 - DNA, 951 bp, Artificial Sequence
  pG1 promoter
  misc_feature (578)..(578): n is (T)x wherein x is 14-16
caaacatttgctccccctagtctccagggaaatgtaaaatatactgctaatagaaaacagtaagacgctcagttgtcaggataattacgttcgactgtagtaaaacaggaatctgtattgttagaaagaacgagagttttttacggcgccgccatattgggccgtgtgaaaacagcttgaaaccccactactttcaaaggttctgttgctatacacgaaccatgtttaaccaacctcgcttttgacttgactgaagtcatcggttaacaatcaagtaccctagtctgtctgaatgctcctttccatattcagtaggtgtttcttgcacttttgcatgcactgcggaagaattagccaatagcgcgtttcatatgcgcttttaccccctcttttgtcaagcgcaaaatgcctgtaagatttggtgggggtgtgagccgttagctgaagtacaacaggctaattccctgaaaaaactgcagatagacttcaagatctcagggattcccactatttggtattctgatatgtttttcctgatatgcatcaaaactctaatctaaaacctgaatctccgctangatgaccccgttttcgtgacaaattaatttccaacggggtcttgtccggataagagaattttgtttgattatccgttcggataaatggacgcctgctccatatttttccggttattaccccacctggaagtgcccagaattttccggggattacggataatacggtggtctggattaattaatacgccaagtcttacattttgttgcagtctcgtgcgagtatgtgcaataataaacaagatgagccaatttattggattagttgcagcttgaccccgccatagctaggcatagccaagtgctatgggtgttagatgatgcacttggatgcagtgagttttggagtataaaagatccttaaaattccaccctt

SEQ ID NO: 46 - DNA, 1238 bp, Artificial Sequence
  pG1-3 promoter
caaacatttgctccccctagtctccagggaaatgtaaaatatactgctaatagaaaacagtaagacgctcagttgtcaggataattacgttcgactgtagtaaaacaggaatctgtattgttagaaagaacgagagttttttacggcgccgccatattgggccgtgtgaaaacagcttgaaaccccactactttcaaaggttctgttgctatacacgaaccatgtttaaccaacctcgcttttgacttgactgaagtcatcggttaacaatcaagtaccctagtctgtctgaatgctcctttccatattcagtaggtgtttcttgcacttttgcatgcactgcggaagaattagccaatagcgcgtttcatatgcgcttttaccccctcttttgtcaagcgcaaaatgcctgtaagatttggtgggggtgtgagccgttagctgaagtacaacaggctaattccctgaaaaaactgcagctcagggattcccactatttggtattctgatatgtttttcctgatatgcatcaaaactctaatctaaaacctgaatctccgctattttttttttttttgatgaccccgttttcgtgacaaattaatttccaacggggtcttgtccggataagagaattttgtttgattatccgttcggataaatggacgcctgctccatatttttccggttattaccccacctggaagtgcccagaattttccggggattacggataatacggtggtctggattaattaatacgagatctcagggattcccactatttggtattctgatatgtttttcctgatatgcatcaaaactctaatctaaaacctgaatctccgctattttttttttttttgatgaccccgttttcgtgacaaattaatttccaacggggtcttgtccggataagagaattttgtttgattatccgttcggataaatggacgcctgctccatatttttccggttattaccccacctggaagtgcccagaattttccggggattacggataatacggtggtctggattaattaatacgccaagtcttacattttgttgcagtctcgtgcgagtatgtgcaataataaacaagatgagccaatttattggattagttgcagcttgaccccgccatagctaggcatagccaagtgctatgggtgttagatgatgcacttggatgcagtgagttttggagtataaaagatccttaaaattccaccctt

SEQ ID NO: 47 - DNA, 1425 bp, Artificial Sequence
  pG1-4 promoter
caaacatttgctccccctagtctccagggaaatgtaaaatatactgctaatagaaaacagtaagacgctcagttgtcaggataattacgttcgactgtagtaaaacaggaatctgtattgttagaaagaacgagagttttttacggcgccgccatattgggccgtgtgaaaacagcttgaaaccccactactttcaaaggttctgttgctatacacgaaccatgtttaaccaacctcgcttttgacttgactgaagtcatcggttaacaatcaagtaccctagtctgtctgaatgctcctttccatattcagtaggtgtttcttgcacttttgcatgcactgcggaagaattagccaatagcgcgtttcatatgcgcttttaccccctcttttgtcaagcgcaaaatgcctgtaagatttggtgggggtgtgagccgttagctgaagtacaacaggctaattccctgaaaaaactgcagctcagggattcccactatttggtattctgatatgtttttcctgatatgcatcaaaactctaatctaaaacctgaatctccgctattttttttttttttgatgaccccgttttcgtgacaaattaatttccaacggggtcttgtccggataagagaattttgtttgattatccgttcggataaatggacgcctgctccatatttttccggttattaccccacctggaagtgcccagaattttccggggattacggataatacggtggtctggattaattaatacgccaagtcttacattttgttgcagtctcgtgcgagtatgtgcaataataaacaagatgagccaatttattggattagttgcagcttgaccccgccatagctaggcatagccaagtgctatgggtgttagatgatgcacttggatgcagtgagttttggagtataaaagatccttaaaattccacccttagatctcagggattcccactatttggtattctgatatgtttttcctgatatgcatcaaaactctaatctaaaacctgaatctccgctattttttttttttttgatgaccccgttttcgtgacaaattaatttccaacggggtcttgtccggataagagaattttgtttgattatccgttcggataaatggacgcctgctccatatttttccggttattaccccacctggaagtgcccagaattttccggggattacggataatacggtggtctggattaattaatacgccaagtcttacattttgttgcagtctcgtgcgagtatgtgcaataataaacaagatgagccaatttattggattagttgcagcttgaccccgccatagctaggcatagccaagtgctatgggtgttagatgatgcacttggatgcagtgagttttggagtataaaagatccttaaaattccaccctt

SEQ ID NO: 48 - protein, 222 aa, Artificial Sequence
  Heavy chain sequence
EVQLVQSGAEVKKPGESLKISCKGSGYSFTSYWIGWVRQMPGKGLEWMGIIYPGDSDTRYSPSFQGQVTISADKSISTAYLQWSSLKASDTAMYYCARFFDADMDSWGQGTLVTVSSASTKGPSVFPLAPSSKSTSGGTAALGCLVKDYFPEPVTVSWNSGALTSGVHTFPAVLQSSGLYSLSSVVTVPSSSLGTQTYICNVNHKPSNTKVDKRVEPKSCDK

SEQ ID NO: 49 - protein, 215 aa, Artificial Sequence
  Light chain sequence
EIVLTQSPATLSLSPGERATLSCGASQSVSSSYLAWYQQKPGLAPRLLIYDASSRATGIPDRFSGSGSGTDFTLTISRLEPEDFAVYYCQQYSNNSVTFGQGTKVEIKRTVAAPSVFIFPPSDEQLKSGTASVVCLLNNFYPREAKVQWKVDNALQSGNSQESVTEQDSKDSTYSLSSTLTLSKADYEKHKVYACEVTHQGLSSPVTKSFNRGEC

SEQ ID NO: 50 - protein, 218 aa, Artificial Sequence
  Heavy chain sequence
DVQLQESGPSLVKPSQTLSLTCSVTGDSITSDYWSWIRKFPGNRLEYMGYVSYSGSTYYNPSLKSRISITRDTSKNQYYLDLNSVTTEDTATYYCANWDGDYWGQGTLVTVSSASTKGPSVFPLAPSSKSTSGGTAALGCLVKDYFPEPVTVSWNSGALTSGVHTFPAVLQSSGLYSLSSVVTVPSSSLGTQTYICNVNHKPSNTKVDKRVEPKSCDK

SEQ ID NO: 51 - protein, 214 aa, Artificial Sequence
  Light chain sequence
DIVLTQSPATLSVTPGNSVSLSCRASQSIGNNLHWYQQKSHESPRLLIKYASQSISGIPSRFSGSGSGTDFTLSINSVETEDFGMYFCQQSNSWPYTFGGGTKLEIKRTVAAPSVFIFPPSDEQLKSGTASVVCLLNNFYPREAKVQWKVDNALQSGNSQESVTEQDSKDSTYSLSSTLTLSKADYEKHKVYACEVTHQGLSSPVTKSFNRGEC

SEQ ID NO: 52 - DNA, 89 bp, Artificial Sequence
  primer
tactaatattacctttacagaattctttccactcctccaatgttttagttagaggtgccgatgatggtagagacttctacaagatcttg